European Patent Application EP 4 464 329 A1, published November 20, 2024. Title: PHARMACEUTICAL COMPOSITION FOR PREVENTING OR TREATING NUERODEGENERATIVE DISEASE COMPRISING GLUCAGON-LIKE PEPTIDE-1 AND IL-1 RECEPTOR ANTAGONIST. Applicant: GI Innovation, Inc. The sequence listing filed with the application follows.

SEQUENCE LISTING (44 sequences)

SEQ ID NO: 1 - protein, 30 aa, synthetic construct
  REGION 1..30: note = hGLP-1
HAEGTFTSDVSSYLEGQAAKEFIAWLVKGR

SEQ ID NO: 2 - protein, 31 aa, synthetic construct
  REGION 1..31: note = hGLP-1 mt-1
HGEGTFTSDVSSYLEEQAAKEFIAWLVKGGG

SEQ ID NO: 3 - protein, 39 aa, synthetic construct
  REGION 1..39: note = hGLP-1 mt-2(exendin-4)
HGEGTFTSDLSKQMEEEAVRLFIEWLKNGGPSSGAPPPS

SEQ ID NO: 4 - protein, 31 aa, synthetic construct
  REGION 1..31: note = hGLP-1 mt-3(liraglutide)
HAEGTFTSDVSSYLEGQAAKEFIAWLVRGRG

SEQ ID NO: 5 - protein, 30 aa, synthetic construct
  REGION 1..30: note = NL028 hinge linker
GGGGSGGGGSGGGGSGGAESKYGPPCPPCP

SEQ ID NO: 6 - protein, 216 aa, synthetic construct
  REGION 1..216: note = hIgG4Fc
APEAAGGPSVFLFPPKPKDQLMISRTPEVTCVVVDVSQEDPEVQFNWYVDGVEVHNAKTKPREEQFNSTYRVVSVLTVLHQDWLNGKEYKCKVSNKGLPSSIEKTISKAKGQPREPQVYTLPPSQEEMTKNQVSLTCLVKGFYPSDIAVEWESNGQPENNYKTTPPVLDSDGSFFLYSRLTVDKSRWQEGNVFSCSVLHEALHNHYTQKSLSLSLG

SEQ ID NO: 7 - protein, 17 aa, synthetic construct
  REGION 1..17: note = (G4S)3GG linker
GGGGSGGGGSGGGGSGG

SEQ ID NO: 8 - protein, 152 aa, synthetic construct
  REGION 1..152: note = IL-1Ra
RPSGRKSSKMQAFRIWDVNQKTFYLRNNQLVAGYLQGPNVNLEEKIDVVPIEPHALFLGIHGGKMCLSCVKSGDETRLQLEAVNITDLSENRKQDKRFAFIRSDSGPTTSFESAACPGWFLCTAMEADQPVSLTNMPDEGVMVTKFYFQEDE

SEQ ID NO: 9 - protein, 19 aa, synthetic construct
  REGION 1..19: note = mIgG signal
MEWSWVFLFFLSVTTGVHS

SEQ ID NO: 10 - protein, 446 aa, synthetic construct
  REGION 1..446: note = GI-210B1(GLP-1-IgG4 Fc-IL-1Ra)
HGEGTFTSDVSSYLEEQAAKEFIAWLVKGGGGGGGSGGGGSGGGGSGGAESKYGPPCPPCPAPEAAGGPSVFLFPPKPKDQLMISRTPEVTCVVVDVSQEDPEVQFNWYVDGVEVHNAKTKPREEQFNSTYRVVSVLTVLHQDWLNGKEYKCKVSNKGLPSSIEKTISKAKGQPREPQVYTLPPSQEEMTKNQVSLTCLVKGFYPSDIAVEWESNGQPENNYKTTPPVLDSDGSFFLYSRLTVDKSRWQEGNVFSCSVLHEALHNHYTQKSLSLSLGGGGGSGGGGSGGGGSGGRPSGRKSSKMQAFRIWDVNQKTFYLRNNQLVAGYLQGPNVNLEEKIDVVPIEPHALFLGIHGGKMCLSCVKSGDETRLQLEAVNITDLSENRKQDKRFAFIRSDSGPTTSFESAACPGWFLCTAMEADQPVSLTNMPDEGVMVTKFYFQEDE

SEQ ID NO: 11 - DNA, 90 bp, synthetic construct
  misc_feature 1..90: note = hGLP-1
  source 1..90: mol_type = other DNA
catgccgagggcacctttacctccgacgtgtcctcctacttggaggaacaggccgccaaagagtttatcgcctggctggtcaaaggtagg

SEQ ID NO: 12 - DNA, 93 bp, synthetic construct
  misc_feature 1..93: note = hGLP-1 mt-1
  source 1..93: mol_type = other DNA
catggcgagggcacctttacctccgacgtgtcctcctacttggaggaacaggccgccaaagagtttatcgcctggctggtcaaaggtggcggc

SEQ ID NO: 13 - DNA, 90 bp, synthetic construct
  misc_feature 1..90: note = NL028 hinge linker
  source 1..90: mol_type = other DNA
ggaggcggaggatccggtggtggtggatctggtggcggaggttctggcggagctgagtctaagtatggccctccttgtcctccatgtcct

SEQ ID NO: 14 - DNA, 648 bp, synthetic construct
  misc_feature 1..648: note = hIgG4Fc
  source 1..648: mol_type = other DNA
gctccagaagctgctggcgggccctccgtgtttctgttccctccaaagcctaaggaccagctgatgatctctcggacccctgaagtgacctgcgtggtggtcgatgtgtcccaagaggaccctgaggtgcagttcaattggtacgtggacggcgtggaagtgcacaacgccaagaccaagcctagagaggaacagttcaactccacctacagagtggtgtccgtgctgaccgtgctgcaccaggattggctgaacggcaaagagtacaagtgcaaggtgtccaacaagggcctgccttccagcatcgaaaagaccatctccaaggccaagggccagcctagggaaccccaggtttacaccctgcctccaagccaagaggaaatgaccaagaaccaggtgtccctgacctgcctggtcaagggcttctacccttccgacattgccgtggaatgggagagcaatggccagcctgagaacaactacaagaccacacctcctgtgctggactccgacggctccttctttctgtactcccgcctgaccgtggacaagtccagatggcaagagggcaacgtgttctcctgctctgtgctgcacgaggccctgcacaatcactacacccagaagtccctcagcctgtcccttgga

SEQ ID NO: 15 - DNA, 51 bp, synthetic construct
  misc_feature 1..51: note = (G4S)3GG linker
  source 1..51: mol_type = other DNA
ggtggtggcggctctggcggtggcggaagtggcggaggtggatccggaggt

SEQ ID NO: 16 - DNA, 456 bp, synthetic construct
  misc_feature 1..456: note = IL-1Ra
  source 1..456: mol_type = other DNA
agaccttctggccggaagtcctctaagatgcaggccttcagaatctgggacgtgaaccagaaaaccttctacctgcggaacaaccagctcgtggccggctatctccagggacctaacgtgaacctggaagagaagatcgacgtggtgcccatcgagccccacgctctgtttttgggaatccacggcggcaagatgtgcctgtcctgtgtgaagtctggcgacgagacacggttgcagctggaagccgtgaacatcaccgacctgtccgagaaccggaagcaggacaagagattcgccttcatcagatccgacagcggccctaccacctccttcgagtctgctgcttgtccaggctggttcctgtgcaccgccatggaagctgaccagcctgtgtctctgaccaacatgcctgacgagggcgtgatggtcaccaagttctacttccaagaggatgag

SEQ ID NO: 17 - DNA, 57 bp, synthetic construct
  misc_feature 1..57: note = mIgG signal
  source 1..57: mol_type = other DNA
atggaatggtcctgggtgttcctgttcttcctgtccgtgaccaccggcgtgcactct

SEQ ID NO: 18 - DNA, 1395 bp, synthetic construct
  misc_feature 1..1395: note = Polynucleotides coding GI-210B1 with signal peptide
  source 1..1395: mol_type = other DNA
atggaatggtcctgggtgttcctgttcttcctgtccgtgaccaccggcgtgcactctcatggcgagggcacctttacctccgacgtgtcctcctacttggaggaacaggccgccaaagagtttatcgcctggctggtcaaaggtggcggcggaggcggaggatccggtggtggtggatctggtggcggaggttctggcggagctgagtctaagtatggccctccttgtcctccatgtcctgctccagaagctgctggcgggccctccgtgtttctgttccctccaaagcctaaggaccagctgatgatctctcggacccctgaagtgacctgcgtggtggtcgatgtgtcccaagaggaccctgaggtgcagttcaattggtacgtggacggcgtggaagtgcacaacgccaagaccaagcctagagaggaacagttcaactccacctacagagtggtgtccgtgctgaccgtgctgcaccaggattggctgaacggcaaagagtacaagtgcaaggtgtccaacaagggcctgccttccagcatcgaaaagaccatctccaaggccaagggccagcctagggaaccccaggtttacaccctgcctccaagccaagaggaaatgaccaagaaccaggtgtccctgacctgcctggtcaagggcttctacccttccgacattgccgtggaatgggagagcaatggccagcctgagaacaactacaagaccacacctcctgtgctggactccgacggctccttctttctgtactcccgcctgaccgtggacaagtccagatggcaagagggcaacgtgttctcctgctctgtgctgcacgaggccctgcacaatcactacacccagaagtccctcagcctgtcccttggaggtggtggcggctctggcggtggcggaagtggcggaggtggatccggaggtagaccttctggccggaagtcctctaagatgcaggccttcagaatctgggacgtgaaccagaaaaccttctacctgcggaacaaccagctcgtggccggctatctccagggacctaacgtgaacctggaagagaagatcgacgtggtgcccatcgagccccacgctctgtttttgggaatccacggcggcaagatgtgcctgtcctgtgtgaagtctggcgacgagacacggttgcagctggaagccgtgaacatcaccgacctgtccgagaaccggaagcaggacaagagattcgccttcatcagatccgacagcggccctaccacctccttcgagtctgctgcttgtccaggctggttcctgtgcaccgccatggaagctgaccagcctgtgtctctgaccaacatgcctgacgagggcgtgatggtcaccaagttctacttccaagaggatgag

SEQ ID NO: 19 - protein, 465 aa, synthetic construct
  REGION 1..465: note = GI-210B1 with signal peptide
MEWSWVFLFFLSVTTGVHSHGEGTFTSDVSSYLEEQAAKEFIAWLVKGGGGGGGSGGGGSGGGGSGGAESKYGPPCPPCPAPEAAGGPSVFLFPPKPKDQLMISRTPEVTCVVVDVSQEDPEVQFNWYVDGVEVHNAKTKPREEQFNSTYRVVSVLTVLHQDWLNGKEYKCKVSNKGLPSSIEKTISKAKGQPREPQVYTLPPSQEEMTKNQVSLTCLVKGFYPSDIAVEWESNGQPENNYKTTPPVLDSDGSFFLYSRLTVDKSRWQEGNVFSCSVLHEALHNHYTQKSLSLSLGGGGGSGGGGSGGGGSGGRPSGRKSSKMQAFRIWDVNQKTFYLRNNQLVAGYLQGPNVNLEEKIDVVPIEPHALFLGIHGGKMCLSCVKSGDETRLQLEAVNITDLSENRKQDKRFAFIRSDSGPTTSFESAACPGWFLCTAMEADQPVSLTNMPDEGVMVTKFYFQEDE

SEQ ID NO: 20 - DNA, 1338 bp, synthetic construct
  misc_feature 1..1338: note = Polynucleotides coding GI-210B1
  source 1..1338: mol_type = other DNA
catggcgagggcacctttacctccgacgtgtcctcctacttggaggaacaggccgccaaagagtttatcgcctggctggtcaaaggtggcggcggaggcggaggatccggtggtggtggatctggtggcggaggttctggcggagctgagtctaagtatggccctccttgtcctccatgtcctgctccagaagctgctggcgggccctccgtgtttctgttccctccaaagcctaaggaccagctgatgatctctcggacccctgaagtgacctgcgtggtggtcgatgtgtcccaagaggaccctgaggtgcagttcaattggtacgtggacggcgtggaagtgcacaacgccaagaccaagcctagagaggaacagttcaactccacctacagagtggtgtccgtgctgaccgtgctgcaccaggattggctgaacggcaaagagtacaagtgcaaggtgtccaacaagggcctgccttccagcatcgaaaagaccatctccaaggccaagggccagcctagggaaccccaggtttacaccctgcctccaagccaagaggaaatgaccaagaaccaggtgtccctgacctgcctggtcaagggcttctacccttccgacattgccgtggaatgggagagcaatggccagcctgagaacaactacaagaccacacctcctgtgctggactccgacggctccttctttctgtactcccgcctgaccgtggacaagtccagatggcaagagggcaacgtgttctcctgctctgtgctgcacgaggccctgcacaatcactacacccagaagtccctcagcctgtcccttggaggtggtggcggctctggcggtggcggaagtggcggaggtggatccggaggtagaccttctggccggaagtcctctaagatgcaggccttcagaatctgggacgtgaaccagaaaaccttctacctgcggaacaaccagctcgtggccggctatctccagggacctaacgtgaacctggaagagaagatcgacgtggtgcccatcgagccccacgctctgtttttgggaatccacggcggcaagatgtgcctgtcctgtgtgaagtctggcgacgagacacggttgcagctggaagccgtgaacatcaccgacctgtccgagaaccggaagcaggacaagagattcgccttcatcagatccgacagcggccctaccacctccttcgagtctgctgcttgtccaggctggttcctgtgcaccgccatggaagctgaccagcctgtgtctctgaccaacatgcctgacgagggcgtgatggtcaccaagttctacttccaagaggatgag

SEQ ID NO: 21 - protein, 9 aa, synthetic construct
  REGION 1..9: note = Additional peptides
PSSGAPPPS

SEQ ID NO: 22 - protein, 277 aa, synthetic construct
  REGION 1..277: note = GLP-1-IgG4 Fc
HGEGTFTSDVSSYLEEQAAKEFIAWLVKGGGGGGGSGGGGSGGGGSGGAESKYGPPCPPCPAPEAAGGPSVFLFPPKPKDQLMISRTPEVTCVVVDVSQEDPEVQFNWYVDGVEVHNAKTKPREEQFNSTYRVVSVLTVLHQDWLNGKEYKCKVSNKGLPSSIEKTISKAKGQPREPQVYTLPPSQEEMTKNQVSLTCLVKGFYPSDIAVEWESNGQPENNYKTTPPVLDSDGSFFLYSRLTVDKSRWQEGNVFSCSVLHEALHNHYTQKSLSLSLG

SEQ ID NO: 23 - DNA, 831 bp, synthetic construct
  misc_feature 1..831: note = Polynucleotides coding GLP-1-IgG4 Fc
  source 1..831: mol_type = other DNA
catggcgagggcacctttacctccgacgtgtcctcctacttggaggaacaggccgccaaagagtttatcgcctggctggtcaaaggtggcggcggaggcggaggatccggtggtggtggatctggtggcggaggttctggcggagctgagtctaagtatggccctccttgtcctccatgtcctgctccagaagctgctggcgggccctccgtgtttctgttccctccaaagcctaaggaccagctgatgatctctcggacccctgaagtgacctgcgtggtggtcgatgtgtcccaagaggaccctgaggtgcagttcaattggtacgtggacggcgtggaagtgcacaacgccaagaccaagcctagagaggaacagttcaactccacctacagagtggtgtccgtgctgaccgtgctgcaccaggattggctgaacggcaaagagtacaagtgcaaggtgtccaacaagggcctgccttccagcatcgaaaagaccatctccaaggccaagggccagcctagggaaccccaggtttacaccctgcctccaagccaagaggaaatgaccaagaaccaggtgtccctgacctgcctggtcaagggcttctacccttccgacattgccgtggaatgggagagcaatggccagcctgagaacaactacaagaccacacctcctgtgctggactccgacggctccttctttctgtactcccgcctgaccgtggacaagtccagatggcaagagggcaacgtgttctcctgctctgtgctgcacgaggccctgcacaatcactacacccagaagtccctcagcctgtcccttgga

SEQ ID NO: 24 - protein, 397 aa, synthetic construct
  REGION 1..385: note = IgG4 Fc-IL-1Ra
ESKYGPPCPPCPAPEAAGGPSVFLFPPKPKDQLMISRTPEVTCVVVDVSQEDPEVQFNWYVDGVEVHNAKTKPREEQFNSTYRVVSVLTVLHQDWLNGKEYKCKVSNKGLPSSIEKTISKAKGQPREPQVYTLPPSQEEMTKNQVSLTCLVKGFYPSDIAVEWESNGQPENNYKTTPPVLDSDGSFFLYSRLTVDKSRWQEGNVFSCSVLHEALHNHYTQKSLSLSLGGGGGSGGGGSGGGGSGGRPSGRKSSKMQAFRIWDVNQKTFYLRNNQLVAGYLQGPNVNLEEKIDVVPIEPHALFLGIHGGKMCLSCVKSGDETRLQLEAVNITDLSENRKQDKRFAFIRSDSGPTTSFESAACPGWFLCTAMEADQPVSLTNMPDEGVMVTKFYFQEDE

SEQ ID NO: 25 - DNA, 1248 bp, synthetic construct
  source 1..1248: mol_type = other DNA
  misc_feature 1..1212: note = Polynucleotides coding IgG4 Fc-IL-1Ra
atggaatggtcctgggtgttcctgttcttcctgtccgtgaccaccggcgtgcactctgaatctaagtacggccctccttgtcctccatgtcctgctccagaagctgctggcgggccctccgtgtttctgttccctccaaagcctaaggaccagctgatgatctctcggacccctgaagtgacctgcgtggtggtcgatgtgtcccaagaggaccctgaggtgcagttcaattggtacgtggacggcgtggaagtgcacaacgccaagaccaagcctagagaggaacagttcaactccacctacagagtggtgtccgtgctgaccgtgctgcaccaggattggctgaacggcaaagagtacaagtgcaaggtgtccaacaagggcctgccttccagcatcgaaaagaccatctccaaggccaagggccagcctagggaaccccaggtttacaccctgcctccaagccaagaggaaatgaccaagaaccaggtgtccctgacctgcctggtcaagggcttctacccttccgacattgccgtggaatgggagagcaatggccagcctgagaacaactacaagaccacacctcctgtgctggactccgacggctccttctttctgtactcccgcctgaccgtggacaagtccagatggcaagagggcaacgtgttctcctgctctgtgctgcacgaggccctgcacaatcactacacccagaagtccctcagcctgtcccttggaggtggtggcggctctggcggtggcggaagtggcggaggtggatccggaggtagaccttctggccggaagtcctctaagatgcaggccttcagaatctgggacgtgaaccagaaaaccttctacctgcggaacaaccagctcgtggccggctatctccagggacctaacgtgaacctggaagagaagatcgacgtggtgcccatcgagccccacgctctgtttttgggaatccacggcggcaagatgtgcctgtcctgtgtgaagtctggcgacgagacacggttgcagctggaagccgtgaacatcaccgacctgtccgagaaccggaagcaggacaagagattcgccttcatcagatccgacagcggccctaccacctccttcgagtctgctgcttgtccaggctggttcctgtgcaccgccatggaagctgaccagcctgtgtctctgaccaacatgcctgacgagggcgtgatggtcaccaagttctacttccaagaggatgag

SEQ ID NO: 26 - protein, 4 aa, synthetic construct
  REGION 1..4: note = GS3
GSSS

SEQ ID NO: 27 - protein, 216 aa, synthetic construct
  REGION 1..216: note = Anti-IL-1 Ab_VH-CH1
QVQLVESGGGVVQPGRSLRLSCAASGFTFSVYGMNWVRQAPGKGLEWVAIIWYDGDNQYYADSVKGRFTISRDNSKNTLYLQMNGLRAEDTAVYYCARDLRTGPFDYWGQGTLVTVSSASTKGPSVFPLAPCSRSTSESTAALGCLVKDYFPEPVTVSWNSGALTSGVHTFPAVLQSSGLYSLSSVVTVPSSSLGTKTYTCNVDHKPSNTKVDKRV

SEQ ID NO: 28 - DNA, 1464 bp, synthetic construct
  source 1..1464: mol_type = other DNA
  misc_feature 1..1464: note = Polynucleotides coding GLP-1-anti-IL-1 Ab-VH-CH1-IgG4 Fc
catggcgagggcacctttacctccgacgtgtcctcctacttggaggaacaggccgccaaagagtttatcgcctggctggtcaaaggcggcggaggatctggcggaggtggaagcggaggcggtggatctcaggttcagctggttgaaagtggcggaggcgttgtgcagcctggcagatctctgagactgtcttgtgccgccagcggcttcaccttctctgtgtacggcatgaactgggtccgacaggctcctggcaaaggcctggaatgggtcgccatcatttggtacgacggcgacaaccagtactacgccgactccgtgaagggcagattcaccatctctcgggacaactccaagaacaccctgtacctccagatgaacggcctgagagccgaggataccgccgtgtactactgtgccagggacctgagaaccggacctttcgattattggggccagggcaccctggtcaccgtgtcctctgcttctaccaagggaccctcggtcttccctctggctccttgctccagatccacctccgagtctacagctgctctgggctgtctggtcaaggactacttccctgagcctgtgaccgtgtcttggaactctggcgctctgacatctggcgtgcacacctttccagctgtgctccagtcctccggcctgtactctctgtctagcgtcgtgaccgtgccttcctctagcctgggcaccaagacctacacctgtaatgtggaccacaagccttccaacaccaaggtggacaagcgcgtggaatctaagtacggccctccttgtcctccatgtcctgctccagaagctgctggcggcccttccgtgtttctgttccctccaaagcctaaggaccagctgatgatctctcggacccctgaagtgacctgcgtggtggtggatgtgtcccaagaggaccctgaggtgcagttcaattggtacgtggacggcgtggaagtgcacaacgccaagaccaagcctagagaggaacagttcaactccacctacagagtggtgtccgtgctgaccgtgctgcaccaggattggctgaacggcaaagagtacaagtgcaaggtgtccaacaagggcctgccttccagcatcgaaaagaccatctctaaggctaagggccagcctcgcgagccccaggtttacacattgcctccaagccaagaggaaatgaccaagaaccaggtgtccctgacctgcctcgtgaagggcttctacccttccgacattgccgtggaatgggagtccaatggccagcctgagaacaactacaagacaacccctcctgtgctggactccgacggctccttctttctgtattcccgcctgaccgtggacaagtctaggtggcaagagggcaacgtgttctcctgctctgtgctgcacgaggccctgcacaatcactacacccagaagtctctgtctctgtccctgggcaag

SEQ ID NO: 29 - protein, 214 aa, synthetic construct
  REGION 1..214: note = Anti-IL-1 Ab_VL-KCL
EIVLTQSPDFQSVTPKEKVTITCRASQSIGSSLHWYQQKPDQSPKLLIKYASQSFSGVPSRFSGSGSGTDFTLTINSLEAEDAAAYYCHQSSSLPFTFGPGTKVDIKRTVAAPSVFIFPPSDEQLKSGTASVVCLLNNFYPREAKVQWKVDNALQSGNSQESVTEQDSKDSTYSLSSTLTLSKADYEKHKVYACEVTHQGLSSPVTKSFNRGEC

SEQ ID NO: 30 - DNA, 642 bp, synthetic construct
  source 1..642: mol_type = other DNA
  misc_feature 1..642: note = Polynucleotides coding Anti-IL-1 Ab_VL-KCL
gagattgtgctgacccagtctcctgacttccagagcgtgacccctaaagagaaagtcaccatcacctgtcgggccagccagtccatcggatcttccctgcattggtatcagcagaagcccgatcagtcccctaagctgctgattaagtacgcctctcagtccttcagcggcgtgccctccagattttctggctctggatctggcaccgacttcaccctgaccatcaactccctggaagccgaggatgccgccgcttactactgtcaccagtcctccagcctgcctttcacctttggacctggcaccaaggtggacatcaagcggacagtggctgccccttccgtgttcatcttcccaccttccgacgagcagctgaagtccggcacagcttctgtcgtgtgcctgctgaacaacttctaccctcgggaagccaaggtgcagtggaaagtggataacgccctccagtccggcaactcccaagagtctgtgaccgagcaggactccaaggacagcacctacagcctgtcctccacactgaccctgtccaaggccgactacgagaagcacaaggtgtacgcctgcgaagtgacccatcagggcctgtctagccctgtgaccaagtctttcaaccggggcgagtgt

SEQ ID NO: 31 - protein, 12 aa, synthetic construct
  REGION 1..12: note = NH06 hinge
ESKYGPPCPPCP

SEQ ID NO: 32 - protein, 118 aa, synthetic construct [sequence omitted]

SEQ ID NO: 33 - protein, 98 aa, synthetic construct
  REGION 1..98: note = Anti-IL-1 Ab_CH1
ASTKGPSVFPLAPCSRSTSESTAALGCLVKDYFPEPVTVSWNSGALTSGVHTFPAVLQSSGLYSLSSVVTVPSSSLGTKTYTCNVDHKPSNTKVDKRV

SEQ ID NO: 34 - protein, 107 aa, synthetic construct [sequence omitted]

SEQ ID NO: 35 - protein, 107 aa, synthetic construct [sequence omitted]

SEQ ID NO: 36 - DNA, 36 bp, synthetic construct
  source 1..36: mol_type = other DNA
  misc_feature 1..36: note = polynucleotide sequence coding NH06 hinge
gaatctaagtacggccctccttgtcctccatgtcct

SEQ ID NO: 37 - protein, 15 aa, synthetic construct
  REGION 1..15: note = (G4S)3 linker
GGGGSGGGGSGGGGS

SEQ ID NO: 38 - protein, 217 aa, synthetic construct
  REGION 1..217: note = hIgG4Fc (F02K)
APEAAGGPSVFLFPPKPKDQLMISRTPEVTCVVVDVSQEDPEVQFNWYVDGVEVHNAKTKPREEQFNSTYRVVSVLTVLHQDWLNGKEYKCKVSNKGLPSSIEKTISKAKGQPREPQVYTLPPSQEEMTKNQVSLTCLVKGFYPSDIAVEWESNGQPENNYKTTPPVLDSDGSFFLYSRLTVDKSRWQEGNVFSCSVLHEALHNHYTQKSLSLSLGK

SEQ ID NO: 39 - protein, 8 aa, synthetic construct
  REGION 1..8: note = HCDR1 of Anti-IL-1
GFTFSVYG

SEQ ID NO: 40 - protein, 8 aa, synthetic construct
  REGION 1..8: note = HCDR2 of anti-IL-1
IWYDGDNQ

SEQ ID NO: 41 - protein, 11 aa, synthetic construct
  REGION 1..11: note = HCDR3 of anti-IL-1
ARDLRTGPFDY

SEQ ID NO: 42 - protein, 6 aa, synthetic construct
  REGION 1..6: note = LCDR1 of Anti-IL-1
QSIGSS

SEQ ID NO: 43 - skipped

SEQ ID NO: 44 - protein, 9 aa, synthetic construct
  REGION 1..9: note = LCDR3 of Anti-IL-1
HQSSSLPFT